European Patent Application EP 4 458 959 A1, published November 6, 2024. Title: Modified Glutamate Dehydrogenase and the Use thereof. Applicant: Hunan Lier Biotech Co., Ltd. The sequence listing filed with the application follows.

SEQUENCE LISTING (80 sequences)

SEQ ID NO: 1 - protein, 457 aa, Bacillus velezensis
MTTTTVSNDQLAKEYVDGVFEQLKNQNSHQAEFLQAAEEIFISLVPVFAQHPEYIKANILSRIVEPDRIISFRVAWQDDNNQVQVNRGYRVQYSNVMGPYKGGLRFHPSVNESIIKFLGFEQIFKNALTGQPIGGGKGGSNFNPKGKSDSEIMRFCQAFMTELYRHIGPDVDVPAGDIGVGAREVGYLWGQYKRITKANESGVLTGKTPGYGGSLARKEATGYGTVYFVEEMLKEVNDSFEDKTVVVSGSGNVSTYAIEKAQAYGAKVVACSDSSGYIYDAEGLDLDVIKEIKEVKGDRISTYVDYRPNATFTEGCTGIWSIPCDIALPCATQNEINGDAARTLISNGVKAIGEGANMPSDLEAINEFLNAGVLFGPAKAANAGGVAVSALEMAQDSSRVFWTFEEVDAKLHQIMKNIYADSKAAADKYGYPGNLVVGANIAGFIKVADGMLAEGIY

SEQ ID NO: 2 - protein, 457 aa, Lysinibacillus sphaericus
MTITTVSNEQLAKEYVDGVFEQLKQQNCHQAEFLQAAEEIFISLVPVFVQHPEYIKANILSRIVEPDRIISFRVAWQDDHNQVQVNRGYRVQYSNVMGPYKGGLRFHPSVNESIIKFLGFEQIFKNALTGQPIGGGKGGSNFDPKGKSDSEIMRFCQAFMTELYRHIGPDVDVPAGDIGVGAREVGYLWGQYKRLTKASESGVLTGKTPGYGGSLARKEATGYGTVYFVNEMLKDVNDSFEGKTVVVSGSGNVSTYAIEKAQQYGAKVVACSDSSGYIYDPEGLDLDVIKEIKEVKGDRISTYVSYRPNATFTNGCTGIWTIPCDIALPCATQNEINGESARTLISNGVKAIGEGANMPSDLEAINEFLNAGVLFGPAKAANAGGVAVSALEMAQDSSRVFWSFEEVDAKLHQIMKDIYSDSKAAAEKYGFPGNLVMGANIAGFIKVADGMLTEGIY

SEQ ID NO: 3 - protein, 457 aa, synthetic construct
MTTTTVSNDQLAKEYVDGVFEQLKNQNSHQAEFLQAAEEIFISLVPVFAQHPEYIKANILSRIVEPDRIISFRVAWQDDNNQVQVNRGYRVQYSNVMGPYKGGLRFHPSVNESIIKFLGFEQIFKNALTGQPIGGGKGGSNFNPKGKSDSEIMRFCQAFMTELYRHIGPDVDVPGGDIGVGAREVGYLWGQYKRITKANESGVLTGKTPGYGGSLARKEATGYGTVYFVEEMLKEVNDSFEDKTVVVSGSGNVSTYAIEKAQAYGAKVVACSDSSGYIYDAEGLDLDVIKEIKEVKGDRISTYVDYRPNATFTEGCTGIWSIPCDIALPCATQNEINGDAARTLISNGVKAIGEGANMPSDLEAINEFLNAGVLFGPAKAANAGGVAVSALEMAQDSSRVFWTFEEVDAKLHQIMKNIYADSKAAADKYGYPGNLVVGANIAGFIKVADGMLAEGIY

SEQ ID NO: 4 - protein, 457 aa, synthetic construct
MTTTTVSNDQLAKEYVDGVFEQLKNQNSHQAEFLQAAEEIFISLVPVFAQHPEYIKANILSRIVEPDRIISFRVAWQDDNNQVQVNRGYRVQYSNVMGPYKGGCRFHPSVNESIIKFLGFEQIFKNALTGQPIGGGKGGSNFNPKGKSDSEIMRFCQAFMTELYRHIGPDVDVPGGDIGVGAREVGYLWGQYKRITKANESGVLTGKTPGYGGSLARKEATGYGTVYFVEEMLKEVNDSFEDKTVVVSGSGNVSTYAIEKAQAYGAKVVACSDSSGYIYDAEGLDLDVIKEIKEVKGDRISTYVDYRPNATFTEGCTGIWSIPCDIALPCATQNEINGDAARTLISNGVKAIGEGANMPSDLEAINEFLNAGVLFGPAKAANAGGVAVSALEMAQDSSRVFWTFEEVDAKLHQIMKNIYADSKAAADKYGYPGNLVVGANIAGFIKVADGMLAEGIY

SEQ ID NO: 5 - protein, 457 aa, synthetic construct
MTTTTVSNDQLAKEYVDGVFEQLKNQNSHQAEFLQAAEEIFISLVPVFAQHPEYIKANILSRIVEPDRIISFRVAWQDDNNQVQVNRGYRVQYSNVMGPYKGGLRFHPSVNESIIKFLGFEQIFKNALTGQLIGGGKGGSNFNPKGKSDSEIMRFCQAFMTELYRHIGPDVDVPGGDIGVGAREVGYLWGQYKRITKANESGVLTGKTPGYGGSLARKEATGYGTVYFVEEMLKEVNDSFEDKTVVVSGSGNVSTYAIEKAQAYGAKVVACSDSSGYIYDAEGLDLDVIKEIKEVKGDRISTYVDYRPNATFTEGCTGIWSIPCDIALPCATQNEINGDAARTLISNGVKAIGEGANMPSDLEAINEFLNAGVLFGPAKAANAGGVAVSALEMAQDSSRVFWTFEEVDAKLHQIMKNIYADSKAAADKYGYPGNLVVGANIAGFIKVADGMLAEGIY

SEQ ID NO: 6 - protein, 457 aa, synthetic construct
MTTTTVSNDQLAKEYVDGVFEQLKNQNSHQAEFLQAAEEIFISLVPVFAQHPEYIKANILSRIVEPDRIISFRVAWQDDNNQVQVNRGYRVQYSNVMGPYKGGLRFHPSVNESIIKFLGFEQIFKNALTGQPVGGGKGGSNFNPKGKSDSEIMRFCQAFMTELYRHIGPDVDVPGGDIGVGAREVGYLWGQYKRITKANESGVLTGKTPGYGGSLARKEATGYGTVYFVEEMLKEVNDSFEDKTVVVSGSGNVSTYAIEKAQAYGAKVVACSDSSGYIYDAEGLDLDVIKEIKEVKGDRISTYVDYRPNATFTEGCTGIWSIPCDIALPCATQNEINGDAARTLISNGVKAIGEGANMPSDLEAINEFLNAGVLFGPAKAANAGGVAVSALEMAQDSSRVFWTFEEVDAKLHQIMKNIYADSKAAADKYGYPGNLVVGANIAGFIKVADGMLAEGIY

SEQ ID NO: 7 - protein, 457 aa, synthetic construct
MTTTTVSNDQLAKEYVDGVFEQLKNQNSHQAEFLQAAEEIFISLVPVFAQHPEYIKANILSRIVEPDRIISFRVAWQDDNNQVQVNRGYRVQYSNVMGPYKGGLRFHPSVNESIIKFLGFEQIFKNALTGQPIGGGKGGSNFNPKGKSDSEIMRFCQAFMTELYRHIGPDVDSPGGDIGVGAREVGYLWGQYKRITKANESGVLTGKTPGYGGSLARKEATGYGTVYFVEEMLKEVNDSFEDKTVVVSGSGNVSTYAIEKAQAYGAKVVACSDSSGYIYDAEGLDLDVIKEIKEVKGDRISTYVDYRPNATFTEGCTGIWSIPCDIALPCATQNEINGDAARTLISNGVKAIGEGANMPSDLEAINEFLNAGVLFGPAKAANAGGVAVSALEMAQDSSRVFWTFEEVDAKLHQIMKNIYADSKAAADKYGYPGNLVVGANIAGFIKVADGMLAEGIY

SEQ ID NO: 8 - protein, 457 aa, synthetic construct
MTTTTVSNDQLAKEYVDGVFEQLKNQNSHQAEFLQAAEEIFISLVPVFAQHPEYIKANILSRIVEPDRIISFRVAWQDDNNQVQVNRGYRVQYSNVMGPYKGGLRFHPSVNESIIKFLGFEQIFKNALTGQPIGGGKGGSNFNPKGKSDSEIMRFCQAFMTELYRHIGPDVDGPGGDIGVGAREVGYLWGQYKRITKANESGVLTGKTPGYGGSLARKEATGYGTVYFVEEMLKEVNDSFEDKTVVVSGSGNVSTYAIEKAQAYGAKVVACSDSSGYIYDAEGLDLDVIKEIKEVKGDRISTYVDYRPNATFTEGCTGIWSIPCDIALPCATQNEINGDAARTLISNGVKAIGEGANMPSDLEAINEFLNAGVLFGPAKAANAGGVAVSALEMAQDSSRVFWTFEEVDAKLHQIMKNIYADSKAAADKYGYPGNLVVGANIAGFIKVADGMLAEGIY

SEQ ID NO: 9 - protein, 457 aa, synthetic construct
MTTTTVSNDQLAKEYVDGVFEQLKNQNSHQAEFLQAAEEIFISLVPVFAQHPEYIKANILSRIVEPDRIISFRVAWQDDNNQVQVNRGYRVQYSNVMGPYKGGLRFHPSVNESIIKFLGFEQIFKNALTGQPIGGGKGGSNFNPKGKSDSEIMRFCQAFMTELYRHIGPDVDVPGGDIGVKAREVGYLWGQYKRITKANESGVLTGKTPGYGGSLARKEATGYGTVYFVEEMLKEVNDSFEDKTVVVSGSGNVSTYAIEKAQAYGAKVVACSDSSGYIYDAEGLDLDVIKEIKEVKGDRISTYVDYRPNATFTEGCTGIWSIPCDIALPCATQNEINGDAARTLISNGVKAIGEGANMPSDLEAINEFLNAGVLFGPAKAANAGGVAVSALEMAQDSSRVFWTFEEVDAKLHQIMKNIYADSKAAADKYGYPGNLVVGANIAGFIKVADGMLAEGIY

SEQ ID NO: 10 - protein, 457 aa, synthetic construct
MTTTTVSNDQLAKEYVDGVFEQLKNQNSHQAEFLQAAEEIFISLVPVFAQHPEYIKANILSRIVEPDRIISFRVAWQDDNNQVQVNRGYRVQYSNVMGPYKGGLRFHPSVNESIIKFLGFEQIFKNALTGQPIGGGKGGSNFNPKGKSDSEIMRFCQAFMTELYRHIGPDVDVPGGDIGVRAREVGYLWGQYKRITKANESGVLTGKTPGYGGSLARKEATGYGTVYFVEEMLKEVNDSFEDKTVVVSGSGNVSTYAIEKAQAYGAKVVACSDSSGYIYDAEGLDLDVIKEIKEVKGDRISTYVDYRPNATFTEGCTGIWSIPCDIALPCATQNEINGDAARTLISNGVKAIGEGANMPSDLEAINEFLNAGVLFGPAKAANAGGVAVSALEMAQDSSRVFWTFEEVDAKLHQIMKNIYADSKAAADKYGYPGNLVVGANIAGFIKVADGMLAEGIY

SEQ ID NO: 11 - protein, 457 aa, synthetic construct
MTTTTVSNDQLAKEYVDGVFEQLKNQNSHQAEFLQAAEEIFISLVPVFAQHPEYIKANILSRIVEPDRIISFRVAWQDDNNQVQVNRGYRVQYSNVMGPYKGGLRFHPSVNESIIKFLGFEQIFKNALTGQPIGGGKGGSNFNPKGKSDSEIMRFCQAFMTELYRHIGPDVDVPGGDIGVGRREVGYLWGQYKRITKANESGVLTGKTPGYGGSLARKEATGYGTVYFVEEMLKEVNDSFEDKTVVVSGSGNVSTYAIEKAQAYGAKVVACSDSSGYIYDAEGLDLDVIKEIKEVKGDRISTYVDYRPNATFTEGCTGIWSIPCDIALPCATQNEINGDAARTLISNGVKAIGEGANMPSDLEAINEFLNAGVLFGPAKAANAGGVAVSALEMAQDSSRVFWTFEEVDAKLHQIMKNIYADSKAAADKYGYPGNLVVGANIAGFIKVADGMLAEGIY

SEQ ID NO: 12 - protein, 457 aa, synthetic construct
MTTTTVSNDQLAKEYVDGVFEQLKNQNSHQAEFLQAAEEIFISLVPVFAQHPEYIKANILSRIVEPDRIISFRVAWQDDNNQVQVNRGYRVQYSNVMGPYKGGLRFHPSVNESIIKFLGFEQIFKNALTGQPIGGGKGGSNFNPKGKSDSEIMRFCQAFMTELYRHIGPDVDVPGGDIGVGAREVGYLWGQYKRITKANESGILTGKTPGYGGSLARKEATGYGTVYFVEEMLKEVNDSFEDKTVVVSGSGNVSTYAIEKAQAYGAKVVACSDSSGYIYDAEGLDLDVIKEIKEVKGDRISTYVDYRPNATFTEGCTGIWSIPCDIALPCATQNEINGDAARTLISNGVKAIGEGANMPSDLEAINEFLNAGVLFGPAKAANAGGVAVSALEMAQDSSRVFWTFEEVDAKLHQIMKNIYADSKAAADKYGYPGNLVVGANIAGFIKVADGMLAEGIY

SEQ ID NO: 13 - protein, 457 aa, synthetic construct
MTTTTVSNDQLAKEYVDGVFEQLKNQNSHQAEFLQAAEEIFISLVPVFAQHPEYIKANILSRIVEPDRIISFRVAWQDDNNQVQVNRGYRVQYSNVMGPYKGGLRFHPSVNESIIKFLGFEQIFKNALTGQLVGGGKGGSNFNPKGKSDSEIMRFCQAFMTELYRHIGPDVDVPGGDIGVGAREVGYLWGQYKRITKANESGVLTGKTPGYGGSLARKEATGYGTVYFVEEMLKEVNDSFEDKTVVVSGSGNVSTYAIEKAQAYGAKVVACSDSSGYIYDAEGLDLDVIKEIKEVKGDRISTYVDYRPNATFTEGCTGIWSIPCDIALPCATQNEINGDAARTLISNGVKAIGEGANMPSDLEAINEFLNAGVLFGPAKAANAGGVAVSALEMAQDSSRVFWTFEEVDAKLHQIMKNIYADSKAAADKYGYPGNLVVGANIAGFIKVADGMLAEGIY

SEQ ID NO: 14 - protein, 457 aa, synthetic construct
MTTTTVSNDQLAKEYVDGVFEQLKNQNSHQAEFLQAAEEIFISLVPVFAQHPEYIKANILSRIVEPDRIISFRVAWQDDNNQVQVNRGYRVQYSNVMGPYKGGLRFHPSVNESIIKFLGFEQIFKNALTGQLIGGGKGGSNFNPKGKSDSEIMRFCQAFMTELYRHIGPDVDSPGGDIGVGAREVGYLWGQYKRITKANESGVLTGKTPGYGGSLARKEATGYGTVYFVEEMLKEVNDSFEDKTVVVSGSGNVSTYAIEKAQAYGAKVVACSDSSGYIYDAEGLDLDVIKEIKEVKGDRISTYVDYRPNATFTEGCTGIWSIPCDIALPCATQNEINGDAARTLISNGVKAIGEGANMPSDLEAINEFLNAGVLFGPAKAANAGGVAVSALEMAQDSSRVFWTFEEVDAKLHQIMKNIYADSKAAADKYGYPGNLVVGANIAGFIKVADGMLAEGIY

SEQ ID NO: 15 - protein, 457 aa, synthetic construct
MTTTTVSNDQLAKEYVDGVFEQLKNQNSHQAEFLQAAEEIFISLVPVFAQHPEYIKANILSRIVEPDRIISFRVAWQDDNNQVQVNRGYRVQYSNVMGPYKGGLRFHPSVNESIIKFLGFEQIFKNALTGQLIGGGKGGSNFNPKGKSDSEIMRFCQAFMTELYRHIGPDVDGPGGDIGVGAREVGYLWGQYKRITKANESGVLTGKTPGYGGSLARKEATGYGTVYFVEEMLKEVNDSFEDKTVVVSGSGNVSTYAIEKAQAYGAKVVACSDSSGYIYDAEGLDLDVIKEIKEVKGDRISTYVDYRPNATFTEGCTGIWSIPCDIALPCATQNEINGDAARTLISNGVKAIGEGANMPSDLEAINEFLNAGVLFGPAKAANAGGVAVSALEMAQDSSRVFWTFEEVDAKLHQIMKNIYADSKAAADKYGYPGNLVVGANIAGFIKVADGMLAEGIY

SEQ ID NO: 16 - protein, 457 aa, synthetic construct
MTTTTVSNDQLAKEYVDGVFEQLKNQNSHQAEFLQAAEEIFISLVPVFAQHPEYIKANILSRIVEPDRIISFRVAWQDDNNQVQVNRGYRVQYSNVMGPYKGGLRFHPSVNESIIKFLGFEQIFKNALTGQLIGGGKGGSNFNPKGKSDSEIMRFCQAFMTELYRHIGPDVDVPGGDIGVGRREVGYLWGQYKRITKANESGVLTGKTPGYGGSLARKEATGYGTVYFVEEMLKEVNDSFEDKTVVVSGSGNVSTYAIEKAQAYGAKVVACSDSSGYIYDAEGLDLDVIKEIKEVKGDRISTYVDYRPNATFTEGCTGIWSIPCDIALPCATQNEINGDAARTLISNGVKAIGEGANMPSDLEAINEFLNAGVLFGPAKAANAGGVAVSALEMAQDSSRVFWTFEEVDAKLHQIMKNIYADSKAAADKYGYPGNLVVGANIAGFIKVADGMLAEGIY

SEQ ID NO: 17 - protein, 457 aa, synthetic construct
MTTTTVSNDQLAKEYVDGVFEQLKNQNSHQAEFLQAAEEIFISLVPVFAQHPEYIKANILSRIVEPDRIISFRVAWQDDNNQVQVNRGYRVQYSNVMGPYKGGLRFHPSVNESIIKFLGFEQIFKNALTGQPVGGGKGGSNFNPKGKSDSEIMRFCQAFMTELYRHIGPDVDSPGGDIGVGAREVGYLWGQYKRITKANESGVLTGKTPGYGGSLARKEATGYGTVYFVEEMLKEVNDSFEDKTVVVSGSGNVSTYAIEKAQAYGAKVVACSDSSGYIYDAEGLDLDVIKEIKEVKGDRISTYVDYRPNATFTEGCTGIWSIPCDIALPCATQNEINGDAARTLISNGVKAIGEGANMPSDLEAINEFLNAGVLFGPAKAANAGGVAVSALEMAQDSSRVFWTFEEVDAKLHQIMKNIYADSKAAADKYGYPGNLVVGANIAGFIKVADGMLAEGIY

SEQ ID NO: 18 - protein, 457 aa, synthetic construct
MTTTTVSNDQLAKEYVDGVFEQLKNQNSHQAEFLQAAEEIFISLVPVFAQHPEYIKANILSRIVEPDRIISFRVAWQDDNNQVQVNRGYRVQYSNVMGPYKGGLRFHPSVNESIIKFLGFEQIFKNALTGQPVGGGKGGSNFNPKGKSDSEIMRFCQAFMTELYRHIGPDVDGPGGDIGVGAREVGYLWGQYKRITKANESGVLTGKTPGYGGSLARKEATGYGTVYFVEEMLKEVNDSFEDKTVVVSGSGNVSTYAIEKAQAYGAKVVACSDSSGYIYDAEGLDLDVIKEIKEVKGDRISTYVDYRPNATFTEGCTGIWSIPCDIALPCATQNEINGDAARTLISNGVKAIGEGANMPSDLEAINEFLNAGVLFGPAKAANAGGVAVSALEMAQDSSRVFWTFEEVDAKLHQIMKNIYADSKAAADKYGYPGNLVVGANIAGFIKVADGMLAEGIY

SEQ ID NO: 19 - protein, 457 aa, synthetic construct
MTTTTVSNDQLAKEYVDGVFEQLKNQNSHQAEFLQAAEEIFISLVPVFAQHPEYIKANILSRIVEPDRIISFRVAWQDDNNQVQVNRGYRVQYSNVMGPYKGGLRFHPSVNESIIKFLGFEQIFKNALTGQPVGGGKGGSNFNPKGKSDSEIMRFCQAFMTELYRHIGPDVDVPGGDIGVGRREVGYLWGQYKRITKANESGVLTGKTPGYGGSLARKEATGYGTVYFVEEMLKEVNDSFEDKTVVVSGSGNVSTYAIEKAQAYGAKVVACSDSSGYIYDAEGLDLDVIKEIKEVKGDRISTYVDYRPNATFTEGCTGIWSIPCDIALPCATQNEINGDAARTLISNGVKAIGEGANMPSDLEAINEFLNAGVLFGPAKAANAGGVAVSALEMAQDSSRVFWTFEEVDAKLHQIMKNIYADSKAAADKYGYPGNLVVGANIAGFIKVADGMLAEGIY

SEQ ID NO: 20 - protein, 457 aa, synthetic construct
MTTTTVSNDQLAKEYVDGVFEQLKNQNSHQAEFLQAAEEIFISLVPVFAQHPEYIKANILSRIVEPDRIISFRVAWQDDNNQVQVNRGYRVQYSNVMGPYKGGLRFHPSVNESIIKFLGFEQIFKNALTGQPIGGGKGGSNFNPKGKSDSEIMRFCQAFMTELYRHIGPDVDSPGGDIGVGRREVGYLWGQYKRITKANESGVLTGKTPGYGGSLARKEATGYGTVYFVEEMLKEVNDSFEDKTVVVSGSGNVSTYAIEKAQAYGAKVVACSDSSGYIYDAEGLDLDVIKEIKEVKGDRISTYVDYRPNATFTEGCTGIWSIPCDIALPCATQNEINGDAARTLISNGVKAIGEGANMPSDLEAINEFLNAGVLFGPAKAANAGGVAVSALEMAQDSSRVFWTFEEVDAKLHQIMKNIYADSKAAADKYGYPGNLVVGANIAGFIKVADGMLAEGIY

SEQ ID NO: 21 - protein, 457 aa, synthetic construct; identical to SEQ ID NO: 8

SEQ ID NO: 22 - protein, 457 aa, synthetic construct
MTTTTVSNDQLAKEYVDGVFEQLKNQNSHQAEFLQAAEEIFISLVPVFAQHPEYIKANILSRIVEPDRIISFRVAWQDDNNQVQVNRGYRVQYSNVMGPYKGGLRFHPSVNESIIKFLGFEQIFKNALTGQLVGGGKGGSNFNPKGKSDSEIMRFCQAFMTELYRHIGPDVDSPGGDIGVGAREVGYLWGQYKRITKANESGVLTGKTPGYGGSLARKEATGYGTVYFVEEMLKEVNDSFEDKTVVVSGSGNVSTYAIEKAQAYGAKVVACSDSSGYIYDAEGLDLDVIKEIKEVKGDRISTYVDYRPNATFTEGCTGIWSIPCDIALPCATQNEINGDAARTLISNGVKAIGEGANMPSDLEAINEFLNAGVLFGPAKAANAGGVAVSALEMAQDSSRVFWTFEEVDAKLHQIMKNIYADSKAAADKYGYPGNLVVGANIAGFIKVADGMLAEGIY

SEQ ID NO: 23 - protein, 457 aa, synthetic construct
MTTTTVSNDQLAKEYVDGVFEQLKNQNSHQAEFLQAAEEIFISLVPVFAQHPEYIKANILSRIVEPDRIISFRVAWQDDNNQVQVNRGYRVQYSNVMGPYKGGLRFHPSVNESIIKFLGFEQIFKNALTGQLVGGGKGGSNFNPKGKSDSEIMRFCQAFMTELYRHIGPDVDGPGGDIGVGAREVGYLWGQYKRITKANESGVLTGKTPGYGGSLARKEATGYGTVYFVEEMLKEVNDSFEDKTVVVSGSGNVSTYAIEKAQAYGAKVVACSDSSGYIYDAEGLDLDVIKEIKEVKGDRISTYVDYRPNATFTEGCTGIWSIPCDIALPCATQNEINGDAARTLISNGVKAIGEGANMPSDLEAINEFLNAGVLFGPAKAANAGGVAVSALEMAQDSSRVFWTFEEVDAKLHQIMKNIYADSKAAADKYGYPGNLVVGANIAGFIKVADGMLAEGIY

SEQ ID NO: 24 - protein, 457 aa, synthetic construct
MTTTTVSNDQLAKEYVDGVFEQLKNQNSHQAEFLQAAEEIFISLVPVFAQHPEYIKANILSRIVEPDRIISFRVAWQDDNNQVQVNRGYRVQYSNVMGPYKGGLRFHPSVNESIIKFLGFEQIFKNALTGQLVGGGKGGSNFNPKGKSDSEIMRFCQAFMTELYRHIGPDVDVPGGDIGVGRREVGYLWGQYKRITKANESGVLTGKTPGYGGSLARKEATGYGTVYFVEEMLKEVNDSFEDKTVVVSGSGNVSTYAIEKAQAYGAKVVACSDSSGYIYDAEGLDLDVIKEIKEVKGDRISTYVDYRPNATFTEGCTGIWSIPCDIALPCATQNEINGDAARTLISNGVKAIGEGANMPSDLEAINEFLNAGVLFGPAKAANAGGVAVSALEMAQDSSRVFWTFEEVDAKLHQIMKNIYADSKAAADKYGYPGNLVVGANIAGFIKVADGMLAEGIY

SEQ ID NO: 25 - protein, 457 aa, synthetic construct
MTTTTVSNDQLAKEYVDGVFEQLKNQNSHQAEFLQAAEEIFISLVPVFAQHPEYIKANILSRIVEPDRIISFRVAWQDDNNQVQVNRGYRVQYSNVMGPYKGGLRFHPSVNESIIKFLGFEQIFKNALTGQLIGGGKGGSNFNPKGKSDSEIMRFCQAFMTELYRHIGPDVDSPGGDIGVGRREVGYLWGQYKRITKANESGVLTGKTPGYGGSLARKEATGYGTVYFVEEMLKEVNDSFEDKTVVVSGSGNVSTYAIEKAQAYGAKVVACSDSSGYIYDAEGLDLDVIKEIKEVKGDRISTYVDYRPNATFTEGCTGIWSIPCDIALPCATQNEINGDAARTLISNGVKAIGEGANMPSDLEAINEFLNAGVLFGPAKAANAGGVAVSALEMAQDSSRVFWTFEEVDAKLHQIMKNIYADSKAAADKYGYPGNLVVGANIAGFIKVADGMLAEGIY

SEQ ID NO: 26 - protein, 457 aa, synthetic construct
MTTTTVSNDQLAKEYVDGVFEQLKNQNSHQAEFLQAAEEIFISLVPVFAQHPEYIKANILSRIVEPDRIISFRVAWQDDNNQVQVNRGYRVQYSNVMGPYKGGLRFHPSVNESIIKFLGFEQIFKNALTGQLIGGGKGGSNFNPKGKSDSEIMRFCQAFMTELYRHIGPDVDGPGGDIGVGRREVGYLWGQYKRITKANESGVLTGKTPGYGGSLARKEATGYGTVYFVEEMLKEVNDSFEDKTVVVSGSGNVSTYAIEKAQAYGAKVVACSDSSGYIYDAEGLDLDVIKEIKEVKGDRISTYVDYRPNATFTEGCTGIWSIPCDIALPCATQNEINGDAARTLISNGVKAIGEGANMPSDLEAINEFLNAGVLFGPAKAANAGGVAVSALEMAQDSSRVFWTFEEVDAKLHQIMKNIYADSKAAADKYGYPGNLVVGANIAGFIKVADGMLAEGIY

SEQ ID NO: 27 - protein, 457 aa, synthetic construct
MTTTTVSNDQLAKEYVDGVFEQLKNQNSHQAEFLQAAEEIFISLVPVFAQHPEYIKANILSRIVEPDRIISFRVAWQDDNNQVQVNRGYRVQYSNVMGPYKGGLRFHPSVNESIIKFLGFEQIFKNALTGQPVGGGKGGSNFNPKGKSDSEIMRFCQAFMTELYRHIGPDVDSPGGDIGVGRREVGYLWGQYKRITKANESGVLTGKTPGYGGSLARKEATGYGTVYFVEEMLKEVNDSFEDKTVVVSGSGNVSTYAIEKAQAYGAKVVACSDSSGYIYDAEGLDLDVIKEIKEVKGDRISTYVDYRPNATFTEGCTGIWSIPCDIALPCATQNEINGDAARTLISNGVKAIGEGANMPSDLEAINEFLNAGVLFGPAKAANAGGVAVSALEMAQDSSRVFWTFEEVDAKLHQIMKNIYADSKAAADKYGYPGNLVVGANIAGFIKVADGMLAEGIY

SEQ ID NO: 28 - protein, 457 aa, synthetic construct
MTTTTVSNDQLAKEYVDGVFEQLKNQNSHQAEFLQAAEEIFISLVPVFAQHPEYIKANILSRIVEPDRIISFRVAWQDDNNQVQVNRGYRVQYSNVMGPYKGGLRFHPSVNESIIKFLGFEQIFKNALTGQPVGGGKGGSNFNPKGKSDSEIMRFCQAFMTELYRHIGPDVDGPGGDIGVGRREVGYLWGQYKRITKANESGVLTGKTPGYGGSLARKEATGYGTVYFVEEMLKEVNDSFEDKTVVVSGSGNVSTYAIEKAQAYGAKVVACSDSSGYIYDAEGLDLDVIKEIKEVKGDRISTYVDYRPNATFTEGCTGIWSIPCDIALPCATQNEINGDAARTLISNGVKAIGEGANMPSDLEAINEFLNAGVLFGPAKAANAGGVAVSALEMAQDSSRVFWTFEEVDAKLHQIMKNIYADSKAAADKYGYPGNLVVGANIAGFIKVADGMLAEGIY

SEQ ID NO: 29 - protein, 457 aa, synthetic construct
MTTTTVSNDQLAKEYVDGVFEQLKNQNSHQAEFLQAAEEIFISLVPVFAQHPEYIKANILSRIVEPDRIISFRVAWQDDNNQVQVNRGYRVQYSNVMGPYKGGLRFHPSVNESIIKFLGFEQIFKNALTGQLVGGGKGGSNFNPKGKSDSEIMRFCQAFMTELYRHIGPDVDSPGGDIGVGRREVGYLWGQYKRITKANESGVLTGKTPGYGGSLARKEATGYGTVYFVEEMLKEVNDSFEDKTVVVSGSGNVSTYAIEKAQAYGAKVVACSDSSGYIYDAEGLDLDVIKEIKEVKGDRISTYVDYRPNATFTEGCTGIWSIPCDIALPCATQNEINGDAARTLISNGVKAIGEGANMPSDLEAINEFLNAGVLFGPAKAANAGGVAVSALEMAQDSSRVFWTFEEVDAKLHQIMKNIYADSKAAADKYGYPGNLVVGANIAGFIKVADGMLAEGIY

SEQ ID NO: 30 - protein, 457 aa, synthetic construct
MTTTTVSNDQLAKEYVDGVFEQLKNQNSHQAEFLQAAEEIFISLVPVFAQHPEYIKANILSRIVEPDRIISFRVAWQDDNNQVQVNRGYRVQYSNVMGPYKGGLRFHPSVNESIIKFLGFEQIFKNALTGQLVGGGKGGSNFNPKGKSDSEIMRFCQAFMTELYRHIGPDVDGPGGDIGVGRREVGYLWGQYKRITKANESGVLTGKTPGYGGSLARKEATGYGTVYFVEEMLKEVNDSFEDKTVVVSGSGNVSTYAIEKAQAYGAKVVACSDSSGYIYDAEGLDLDVIKEIKEVKGDRISTYVDYRPNATFTEGCTGIWSIPCDIALPCATQNEINGDAARTLISNGVKAIGEGANMPSDLEAINEFLNAGVLFGPAKAANAGGVAVSALEMAQDSSRVFWTFEEVDAKLHQIMKNIYADSKAAADKYGYPGNLVVGANIAGFIKVADGMLAEGIY

SEQ ID NO: 31 - protein, 457 aa, synthetic construct
MTITTVSNEQLAKEYVDGVFEQLKQQNCHQAEFLQAAEEIFISLVPVFVQHPEYIKANILSRIVEPDRIISFRVAWQDDHNQVQVNRGYRVQYSNVMGPYKGGLRFHPSVNESIIKFLGFEQIFKNALTGQPIGGGKGGSNFDPKGKSDSEIMRFCQAFMTELYRHIGPDVDVPGGDIGVGAREVGYLWGQYKRLTKASESGVLTGKTPGYGGSLARKEATGYGTVYFVNEMLKDVNDSFEGKTVVVSGSGNVSTYAIEKAQQYGAKVVACSDSSGYIYDPEGLDLDVIKEIKEVKGDRISTYVSYRPNATFTNGCTGIWTIPCDIALPCATQNEINGESARTLISNGVKAIGEGANMPSDLEAINEFLNAGVLFGPAKAANAGGVAVSALEMAQDSSRVFWSFEEVDAKLHQIMKDIYSDSKAAAEKYGFPGNLVMGANIAGFIKVADGMLTEGIY

SEQ ID NO: 32 - protein, 457 aa, synthetic construct
MTITTVSNEQLAKEYVDGVFEQLKQQNCHQAEFLQAAEEIFISLVPVFVQHPEYIKANILSRIVEPDRIISFRVAWQDDHNQVQVNRGYRVQYSNVMGPYKGGLRFHPSVNESIIKFLGFEQIFKNALTGQLIGGGKGGSNFDPKGKSDSEIMRFCQAFMTELYRHIGPDVDVPGGDIGVGAREVGYLWGQYKRLTKASESGVLTGKTPGYGGSLARKEATGYGTVYFVNEMLKDVNDSFEGKTVVVSGSGNVSTYAIEKAQQYGAKVVACSDSSGYIYDPEGLDLDVIKEIKEVKGDRISTYVSYRPNATFTNGCTGIWTIPCDIALPCATQNEINGESARTLISNGVKAIGEGANMPSDLEAINEFLNAGVLFGPAKAANAGGVAVSALEMAQDSSRVFWSFEEVDAKLHQIMKDIYSDSKAAAEKYGFPGNLVMGANIAGFIKVADGMLTEGIY

SEQ ID NO: 33 - protein, 457 aa, synthetic construct; identical to SEQ ID NO: 32

SEQ ID NO: 34 - protein, 457 aa, synthetic construct
MTITTVSNEQLAKEYVDGVFEQLKQQNCHQAEFLQAAEEIFISLVPVFVQHPEYIKANILSRIVEPDRIISFRVAWQDDHNQVQVNRGYRVQYSNVMGPYKGGLRFHPSVNESIIKFLGFEQIFKNALTGQPIGGGKGGSNFDPKGKSDSEIMRFCQAFMTELYRHIGPDVDSPGGDIGVGAREVGYLWGQYKRLTKASESGVLTGKTPGYGGSLARKEATGYGTVYFVNEMLKDVNDSFEGKTVVVSGSGNVSTYAIEKAQQYGAKVVACSDSSGYIYDPEGLDLDVIKEIKEVKGDRISTYVSYRPNATFTNGCTGIWTIPCDIALPCATQNEINGESARTLISNGVKAIGEGANMPSDLEAINEFLNAGVLFGPAKAANAGGVAVSALEMAQDSSRVFWSFEEVDAKLHQIMKDIYSDSKAAAEKYGFPGNLVMGANIAGFIKVADGMLTEGIY

SEQ ID NO: 35 - protein, 457 aa, synthetic construct
MTITTVSNEQLAKEYVDGVFEQLKQQNCHQAEFLQAAEEIFISLVPVFVQHPEYIKANILSRIVEPDRIISFRVAWQDDHNQVQVNRGYRVQYSNVMGPYKGGLRFHPSVNESIIKFLGFEQIFKNALTGQPIGGGKGGSNFDPKGKSDSEIMRFCQAFMTELYRHIGPDVDGPGGDIGVGAREVGYLWGQYKRLTKASESGVLTGKTPGYGGSLARKEATGYGTVYFVNEMLKDVNDSFEGKTVVVSGSGNVSTYAIEKAQQYGAKVVACSDSSGYIYDPEGLDLDVIKEIKEVKGDRISTYVSYRPNATFTNGCTGIWTIPCDIALPCATQNEINGESARTLISNGVKAIGEGANMPSDLEAINEFLNAGVLFGPAKAANAGGVAVSALEMAQDSSRVFWSFEEVDAKLHQIMKDIYSDSKAAAEKYGFPGNLVMGANIAGFIKVADGMLTEGIY

SEQ ID NO: 36 - protein, 457 aa, synthetic construct
MTITTVSNEQLAKEYVDGVFEQLKQQNCHQAEFLQAAEEIFISLVPVFVQHPEYIKANILSRIVEPDRIISFRVAWQDDHNQVQVNRGYRVQYSNVMGPYKGGLRFHPSVNESIIKFLGFEQIFKNALTGQPIGGGKGGSNFDPKGKSDSEIMRFCQAFMTELYRHIGPDVDVPGGDIGVGRREVGYLWGQYKRLTKASESGVLTGKTPGYGGSLARKEATGYGTVYFVNEMLKDVNDSFEGKTVVVSGSGNVSTYAIEKAQQYGAKVVACSDSSGYIYDPEGLDLDVIKEIKEVKGDRISTYVSYRPNATFTNGCTGIWTIPCDIALPCATQNEINGESARTLISNGVKAIGEGANMPSDLEAINEFLNAGVLFGPAKAANAGGVAVSALEMAQDSSRVFWSFEEVDAKLHQIMKDIYSDSKAAAEKYGFPGNLVMGANIAGFIKVADGMLTEGIY

SEQ ID NO: 37 - protein, 457 aa, synthetic construct
MTITTVSNEQLAKEYVDGVFEQLKQQNCHQAEFLQAAEEIFISLVPVFVQHPEYIKANILSRIVEPDRIISFRVAWQDDHNQVQVNRGYRVQYSNVMGPYKGGLRFHPSVNESIIKFLGFEQIFKNALTGQPIGGGKGGSNFDPKGKSDSEIMRFCQAFMTELYRHIGPDVDGPGGDIGVGRREVGYLWGQYKRLTKASESGVLTGKTPGYGGSLARKEATGYGTVYFVNEMLKDVNDSFEGKTVVVSGSGNVSTYAIEKAQQYGAKVVACSDSSGYIYDPEGLDLDVIKEIKEVKGDRISTYVSYRPNATFTNGCTGIWTIPCDIALPCATQNEINGESARTLISNGVKAIGEGANMPSDLEAINEFLNAGVLFGPAKAANAGGVAVSALEMAQDSSRVFWSFEEVDAKLHQIMKDIYSDSKAAAEKYGFPGNLVMGANIAGFIKVADGMLTEGIY

SEQ ID NO: 38 - protein, 457 aa, synthetic construct
MTITTVSNEQLAKEYVDGVFEQLKQQNCHQAEFLQAAEEIFISLVPVFVQHPEYIKANILSRIVEPDRIISFRVAWQDDHNQVQVNRGYRVQYSNVMGPYKGGLRFHPSVNESIIKFLGFEQVFKNALTGQPIGGGKGGSNFDPKGKSDSEIMRFCQAFMTELYRHIGPDVDSPGGDIGVGRREVGYLWGQYKRLTKASESGVLTGKTPGYGGSLARKEATGYGTVYFVNEMLKDVNDSFEGKTVVVSGSGNVSTYAIEKAQQYGAKVVACSDSSGYIYDPEGLDLDVIKEIKEVKGDRISTYVSYRPNATFTNGCTGIWTIPCDIALPCATQNEINGESARTLISNGVKAIGEGANMPSDLEAINEFLNAGVLFGPAKAANAGGVAVSALEMAQDSSRVFWSFEEVDAKLHQIMKDIYSDSKAAAEKYGFPGNLVMGANIAGFIKVADGMLTEGIY

SEQ ID NO: 39 - protein, 457 aa, synthetic construct; identical to SEQ ID NO: 8

SEQ ID NO: 40 - protein, 457 aa, synthetic construct
MTTTTVSNDQLAKEYVDGVFEELKNQNSHQAEFLQAAEEIFISLVPVFAQHPEYIKANILSRIVEPDRIISFRVAWQDDNNQVQVNRGYRVQYSNVMGPYKGGLRFHPSVNESIIKFLGFEQIFKNALTGQPIGGGKGGSNFNPKGKSDSEIMRFCQAFMTELYRHIGPDVDGPGGDIGVGAREVGYLWGQYKRITKANESGVLTGKTPGYGGSLARKEATGYGTVYFVEEMLKEVNDSFEDKTVVVSGSGNVSTYAIEKAQAYGAKVVACSDSSGYIYDAEGLDLDVIKEIKEVKGDRISTYVDYRPNATFTEGCTGIWSIPCDIALPCATQNEINGDAARTLISNGVKAIGEGANMPSDLEAINEFLNAGVLFGPAKAANAGGVAVSALEMAQDSSRVFWTFEEVDAKLHQIMKNIYADSKAAADKYGYPGNLVVGANIAGFIKVADGMLAEGIY

SEQ ID NO: 41 - protein, 457 aa, synthetic construct
MTTTTVSNDQLAKEYVDGVFEQMKNQNSHQAEFLQAAEEIFISLVPVFAQHPEYIKANILSRIVEPDRIISFRVAWQDDNNQVQVNRGYRVQYSNVMGPYKGGLRFHPSVNESIIKFLGFEQIFKNALTGQPIGGGKGGSNFNPKGKSDSEIMRFCQAFMTELYRHIGPDVDGPGGDIGVGAREVGYLWGQYKRITKANESGVLTGKTPGYGGSLARKEATGYGTVYFVEEMLKEVNDSFEDKTVVVSGSGNVSTYAIEKAQAYGAKVVACSDSSGYIYDAEGLDLDVIKEIKEVKGDRISTYVDYRPNATFTEGCTGIWSIPCDIALPCATQNEINGDAARTLISNGVKAIGEGANMPSDLEAINEFLNAGVLFGPAKAANAGGVAVSALEMAQDSSRVFWTFEEVDAKLHQIMKNIYADSKAAADKYGYPGNLVVGANIAGFIKVADGMLAEGIY

SEQ ID NO: 42 - protein, 457 aa, synthetic construct
MTTTTVSNDQLAKEYVDGVFEQLKNQNSHQAEFLQAAEEIFISLVPVFAQHPEYIQANILSRIVEPDRIISFRVAWQDDNNQVQVNRGYRVQYSNVMGPYKGGLRFHPSVNESIIKFLGFEQIFKNALTGQPIGGGKGGSNFNPKGKSDSEIMRFCQAFMTELYRHIGPDVDGPGGDIGVGAREVGYLWGQYKRITKANESGVLTGKTPGYGGSLARKEATGYGTVYFVEEMLKEVNDSFEDKTVVVSGSGNVSTYAIEKAQAYGAKVVACSDSSGYIYDAEGLDLDVIKEIKEVKGDRISTYVDYRPNATFTEGCTGIWSIPCDIALPCATQNEINGDAARTLISNGVKAIGEGANMPSDLEAINEFLNAGVLFGPAKAANAGGVAVSALEMAQDSSRVFWTFEEVDAKLHQIMKNIYADSKAAADKYGYPGNLVVGANIAGFIKVADGMLAEGIY

SEQ ID NO: 43 - protein, 457 aa, synthetic construct
MTTTTVSNSQLAKEYVDGVFEQLKNQNSHQAEFLQAAEEIFISLVPVFAQHPEYIKANILSRIVEPDRIISFRVAWQDDNNQVQVNRGYRVQYSNVMGPYKGGLRFHPSVNESIIKFLGFEQIFKNALTGQPIGGGKGGSNFNPKGKSDSEIMRFCQAFMTELYRHIGPDVDGPGGDIGVGAREVGYLWGQYKRITKANESGVLTGKTPGYGGSLARKEATGYGTVYFVEEMLKEVNDSFEDKTVVVSGSGNVSTYAIEKAQAYGAKVVACSDSSGYIYDAEGLDLDVIKEIKEVKGDRISTYVDYRPNATFTEGCTGIWSIPCDIALPCATQNEINGDAARTLISNGVKAIGEGANMPSDLEAINEFLNAGVLFGPAKAANAGGVAVSALEMAQDSSRVFWTFEEVDAKLHQIMKNIYADSKAAADKYGYPGNLVVGANIAGFIKVADGMLAEGIY

SEQ ID NO: 44 - protein, 457 aa, synthetic construct
MTTTTVSNLQLAKEYVDGVFEQLKNQNSHQAEFLQAAEEIFISLVPVFAQHPEYIKANILSRIVEPDRIISFRVAWQDDNNQVQVNRGYRVQYSNVMGPYKGGLRFHPSVNESIIKFLGFEQIFKNALTGQPIGGGKGGSNFNPKGKSDSEIMRFCQAFMTELYRHIGPDVDGPGGDIGVGAREVGYLWGQYKRITKANESGVLTGKTPGYGGSLARKEATGYGTVYFVEEMLKEVNDSFEDKTVVVSGSGNVSTYAIEKAQAYGAKVVACSDSSGYIYDAEGLDLDVIKEIKEVKGDRISTYVDYRPNATFTEGCTGIWSIPCDIALPCATQNEINGDAARTLISNGVKAIGEGANMPSDLEAINEFLNAGVLFGPAKAANAGGVAVSALEMAQDSSRVFWTFEEVDAKLHQIMKNIYADSKAAADKYGYPGNLVVGANIAGFIKVADGMLAEGIY

SEQ ID NO: 45 - protein, 457 aa, synthetic construct
MTTTTVSNYQLAKEYVDGVFEQLKNQNSHQAEFLQAAEEIFISLVPVFAQHPEYIKANILSRIVEPDRIISFRVAWQDDNNQVQVNRGYRVQYSNVMGPYKGGLRFHPSVNESIIKFLGFEQIFKNALTGQPIGGGKGGSNFNPKGKSDSEIMRFCQAFMTELYRHIGPDVDGPGGDIGVGAREVGYLWGQYKRITKANESGVLTGKTPGYGGSLARKEATGYGTVYFVEEMLKEVNDSFEDKTVVVSGSGNVSTYAIEKAQAYGAKVVACSDSSGYIYDAEGLDLDVIKEIKEVKGDRISTYVDYRPNATFTEGCTGIWSIPCDIALPCATQNEINGDAARTLISNGVKAIGEGANMPSDLEAINEFLNAGVLFGPAKAANAGGVAVSALEMAQDSSRVFWTFEEVDAKLHQIMKNIYADSKAAADKYGYPGNLVVGANIAGFIKVADGMLAEGIY

SEQ ID NO: 46 - protein, 457 aa, synthetic construct
MTTTTVSNDQLAKEYVDGVFEQLKDQNSHQAEFLQAAEEIFISLVPVFAQHPEYIKANILSRIVEPDRIISFRVAWQDDNNQVQVNRGYRVQYSNVMGPYKGGLRFHPSVNESIIKFLGFEQIFKNALTGQPIGGGKGGSNFNPKGKSDSEIMRFCQAFMTELYRHIGPDVDGPGGDIGVGAREVGYLWGQYKRITKANESGVLTGKTPGYGGSLARKEATGYGTVYFVEEMLKEVNDSFEDKTVVVSGSGNVSTYAIEKAQAYGAKVVACSDSSGYIYDAEGLDLDVIKEIKEVKGDRISTYVDYRPNATFTEGCTGIWSIPCDIALPCATQNEINGDAARTLISNGVKAIGEGANMPSDLEAINEFLNAGVLFGPAKAANAGGVAVSALEMAQDSSRVFWTFEEVDAKLHQIMKNIYADSKAAADKYGYPGNLVVGANIAGFIKVADGMLAEGIY

SEQ ID NO: 47 - protein, 457 aa, synthetic construct
MTTTTVSNDQLAKEYVDGVFEQLKNQNSHQAEFLQAAEEIFISLVPVFAQHPEYIKANILSRIVEPDRIISFRVAWQDDNNQVQVNRGYRVQYSNVMGPYKGGLRFHPSVNESIIKFLGFEQIFKNALTGQPIGGGKGGSNFNPKGKSDSEIMRFCQAFMTELYRHIGPDVDGPGGDIGVGAREVGYLWGQYKRITKAWESGVLTGKTPGYGGSLARKEATGYGTVYFVEEMLKEVNDSFEDKTVVVSGSGNVSTYAIEKAQAYGAKVVACSDSSGYIYDAEGLDLDVIKEIKEVKGDRISTYVDYRPNATFTEGCTGIWSIPCDIALPCATQNEINGDAARTLISNGVKAIGEGANMPSDLEAINEFLNAGVLFGPAKAANAGGVAVSALEMAQDSSRVFWTFEEVDAKLHQIMKNIYADSKAAADKYGYPGNLVVGANIAGFIKVADGMLAEGIY

SEQ ID NO: 48 - protein, 457 aa, synthetic construct
MTTTTVSNDQLAKEYVDGVFEQLKNQNSHQAEFLQAAEEIFISLVPVFAQHPEYIKANILSRIVEPDRIISFRVAWQDDNNQVQVNRGYRVQYSNVMGPYKGGLRFHPSVNESIIKFLGFEQIFKNALTGQPIGGGKGGSNFNPKGKSDSEIMRFCQAFMTELYRHIGPDVDGPGGDIGVGAREVGYLWGQYKRITKAYESGVLTGKTPGYGGSLARKEATGYGTVYFVEEMLKEVNDSFEDKTVVVSGSGNVSTYAIEKAQAYGAKVVACSDSSGYIYDAEGLDLDVIKEIKEVKGDRISTYVDYRPNATFTEGCTGIWSIPCDIALPCATQNEINGDAARTLISNGVKAIGEGANMPSDLEAINEFLNAGVLFGPAKAANAGGVAVSALEMAQDSSRVFWTFEEVDAKLHQIMKNIYADSKAAADKYGYPGNLVVGANIAGFIKVADGMLAEGIY

SEQ ID NO: 49 - protein, 457 aa, synthetic construct
MTTTTVSNDQLAKEYVDGVFEQLKNQNSHQAEFLQAAEEIFISLVPVFAQHPEYIKANILSRIVEPDRIISFRVAWQDDNNQVQVNRGYRVQYSNVMGPYKGGLRFHPSVNESIIKFLGFEQIFKNALTGQPIGGGKGGSNFNPKGKSDSEIMRFCQAFMTELYRHIGPDVDGPGGDIGVGAREVGYLWGQYKRITKANESGVLTGKTPGYGGSLARKEATGYGTVYFVEEMLKEVNDSFEGKTVVVSGSGNVSTYAIEKAQAYGAKVVACSDSSGYIYDAEGLDLDVIKEIKEVKGDRISTYVDYRPNATFTEGCTGIWSIPCDIALPCATQNEINGDAARTLISNGVKAIGEGANMPSDLEAINEFLNAGVLFGPAKAANAGGVAVSALEMAQDSSRVFWTFEEVDAKLHQIMKNIYADSKAAADKYGYPGNLVVGANIAGFIKVADGMLAEGIY

SEQ ID NO: 50 - protein, 457 aa, synthetic construct
MTTTTVSNDQLAKEYVDGVFEQLKNQNSHQAEFLQAAEEIFISLVPVFAQHPEYIKANILSRIVEPDRIISFRVAWQDDNNQVQVNRGYRVQYSNVMGPYKGGLRFHPSVNESIIKFLGFEQIFKNALTGQPIGGGKGGSNFEPKGKSDSEIMRFCQAFMTELYRHIGPDVDGPGGDIGVGAREVGYLWGQYKRITKANESGVLTGKTPGYGGSLARKEATGYGTVYFVEEMLKEVNDSFEDKTVVVSGSGNVSTYAIEKAQAYGAKVVACSDSSGYIYDAEGLDLDVIKEIKEVKGDRISTYVDYRPNATFTEGCTGIWSIPCDIALPCATQNEINGDAARTLISNGVKAIGEGANMPSDLEAINEFLNAGVLFGPAKAANAGGVAVSALEMAQDSSRVFWTFEEVDAKLHQIMKNIYADSKAAADKYGYPGNLVVGANIAGFIKVADGMLAEGIY

SEQ ID NO: 51 - protein, 457 aa, synthetic construct
MTTTTVSNDQLAKEYVDGVFEQLKNQNSHQAEFLQAAEEIFISLVPVFAQHPEYIKANILSRIVEPDRIISFRVAWQDDNNQVQVNRGYRVQYSNVMGPYKGGLRFHPSVNESIIKFLGFEQIFKNALTGQPIGGGKGGSNFNPKGKSDSEIMRFCQAFMTELYRHIGPDVDGPGGDIGVGAREVGYLWGQYKRITKANESGVLTGKTPGYGGSLARKEATGYGTVYFVEEMLKEVNDSFEDKTVVVSGSGNVSTYAIEKAQSYGAKVVACSDSSGYIYDAEGLDLDVIKEIKEVKGDRISTYVDYRPNATFTEGCTGIWSIPCDIALPCATQNEINGDAARTLISNGVKAIGEGANMPSDLEAINEFLNAGVLFGPAKAANAGGVAVSALEMAQDSSRVFWTFEEVDAKLHQIMKNIYADSKAAADKYGYPGNLVVGANIAGFIKVADGMLAEGIY

SEQ ID NO: 52 - protein, 457 aa, synthetic construct
MTTTTVSNDQLAKEYVDGVFEQLKNQNSHQAEFLQAAEEIFISLVPVFAQHPEYIKANILSRIVEPDRIISFRVAWQDDNNQVQVNRGYRVQYSNVMGPYKGGLRFHPSVNESIIKFLGFEQIFKNALTGQPIGGGKGGSNFNPKGKSDSEIMRFCQAFMTELYRHIGPDVDGPGGDIGVGAREVGYLWGQYKRITKANESGVLTGKTPGYGGSLARKEATGYGTVYFVEEMLKEVNDSFEDKTVVVSGSGNVSTYAIEKAQKYGAKVVACSDSSGYIYDAEGLDLDVIKEIKEVKGDRISTYVDYRPNATFTEGCTGIWSIPCDIALPCATQNEINGDAARTLISNGVKAIGEGANMPSDLEAINEFLNAGVLFGPAKAANAGGVAVSALEMAQDSSRVFWTFEEVDAKLHQIMKNIYADSKAAADKYGYPGNLVVGANIAGFIKVADGMLAEGIY

SEQ ID NO: 53 - protein, 457 aa, synthetic construct
MTTTTVSNDQLAKEYVDGVFEQLKNQNSHQAEFLQAAEEIFISLVPVFAQHPEYIKANILSRIVEPDRIISFRVAWQDDNNQVQVNRGYRVQYSNVMGPYKGGLRFHPSVNESIIKFLGFEQIFKNALTGQPIGGGKGGSNFNPKGKSDSEIMRFCQAFMTELYRHIGPDVDGPGGDIGVGAREVGYLWGQYKRITKANESGVLTGKTPGYGGSLARKEATGYGTVYFVEEMLKEVNDSFEDKTVVVSGSGNVSTYAIEKAQAYGAKVVACSDSSGYIYDAEGLDLDVIKEIKEVKGDRISTYVDYRPNATFTEGCTGIWSIPCDIALPCATQNEINGQAARTLISNGVKAIGEGANMPSDLEAINEFLNAGVLFGPAKAANAGGVAVSALEMAQDSSRVFWTFEEVDAKLHQIMKNIYADSKAAADKYGYPGNLVVGANIAGFIKVADGMLAEGIY

SEQ ID NO: 54 - protein, 457 aa, synthetic construct
MTTTTVSNDQLAKEYVDGVFEQLKNQNSHQAEFLQAAEEIFISLVPVFAQHPEYIKANILSRIVEPDRIISFRVAWQDDNNQVQVNRGYRVQYSNVMGPYKGGLRFHPSVNESIIKFLGFEQIFKNALTGQPIGGGKGGSNFNPKGKSDSEIMRFCQAFMTELYRHIGPDVDGPGGDIGVGAREVGYLWGQYKRITKANESGVLTGKTPGYGGSLARKEATGYGTVYFVEEMLKEVNDSFEDKTVVVSGSGNVSTYAIEKAQAYGAKVVACSDSSGYIYDAEGLDLDVIKEIKEVKGDRISTYVDYRPNATFTEGCTGIWSIPCDIALPCATQNEINGDAARTLISNGVKAIGEGANMPSDLEAINEFLNAGVLFGPAKAANAGGVAVSALEMAQDSSRVFWTFEEVDAKLHQIMKNIYRDSKAAADKYGYPGNLVVGANIAGFIKVADGMLAEGIY

SEQ ID NO: 55 - protein, 457 aa, synthetic construct
MTTTTVSNDQLAKEYVDGVFEQLKNQNSHQAEFLQAAEEIFISLVPVFAQHPEYIKANILSRIVEPDRIISFRVAWQDDNNQVQVNRGYRVQYSNVMGPYKGGLRFHPSVNESIIKFLGFEQIFKNALTGQPIGGGKGGSNFNPKGKSDSEIMRFCQAFMTELYRHIGPDVDGPGGDIGVGAREVGYLWGQYKRITKANESGVLTGKTPGYGGSLARKEATGYGTVYFVEEMLKEVNDSFEDKTVVVSGSGNVSTYAIEKAQAYGAKVVACSDSSGYIYDAEGLDLDVIKEIKEVKGDRISTYVDYRPNATFTEGCTGIWSIPCDIALPCATQNEINGDAARTLISNGVKAIGEGANMPSDLEAINEFLNAGVLFGPAKAANAGGVAVSALEMAQDSSRVFWTFEEVDAKLHQIMKNIYADSKAAADKYGSPGNLVVGANIAGFIKVADGMLAEGIY

SEQ ID NO: 56 - protein, 457 aa, synthetic construct
MTTTTVSNDQLAKEYVDGVFEQLKNQNSHQAEFLQAAEEIFISLVPVFAQHPEYIKANILSRIVEPDRIISFRVAWQDDNNQVQVNRGYRVQYSNVMGPYKGGLRFHPSVNESIIKFLGFEQIFKNALTGQPIGGGKGGSNFNPKGKSDSEIMRFCQAFMTELYRHIGPDVDGPGGDIGVGAREVGYLWGQYKRITKANESGVLTGKTPGYGGSLARKEATGYGTVYFVEEMLKEVNDSFEDKTVVVSGSGNVSTYAIEKAQAYGAKVVACSDSSGYIYDAEGLDLDVIKEIKEVKGDRISTYVDYRPNATFTEGCTGIWSIPCDIALPCATQNEINGDAARTLISNGVKAIGEGANMPSDLEAINEFLNAGVLFGPAKAANAGGVAVSALEMAQDSSRVFWTFEEVDAKLHQIMKNIYADSKAAADKYGYPGNLVKGANIAGFIKVADGMLAEGIY

SEQ ID NO: 57 - protein, 457 aa, synthetic construct
MTTTTVSNDQLAKEYVDGVFEQLKNQNSHQAEFLQAAEEIFISLVPVFAQHPEYIQANILSRIVEPDRIISFRVAWQDDNNQVQVNRGYRVQYSNVMGPYKGGLRFHPSVNESIIKFLGFEQIFKNALTGQPIGGGKGGSNFNPKGKSDSEIMRFCQAFMTELYRHIGPDVDGPGGDIGVGAREVGYLWGQYKRITKAWESGVLTGKTPGYGGSLARKEATGYGTVYFVEEMLKEVNDSFEDKTVVVSGSGNVSTYAIEKAQAYGAKVVACSDSSGYIYDAEGLDLDVIKEIKEVKGDRISTYVDYRPNATFTEGCTGIWSIPCDIALPCATQNEINGDAARTLISNGVKAIGEGANMPSDLEAINEFLNAGVLFGPAKAANAGGVAVSALEMAQDSSRVFWTFEEVDAKLHQIMKNIYADSKAAADKYGYPGNLVVGANIAGFIKVADGMLAEGIY

SEQ ID NO: 58 - protein, 457 aa, synthetic construct
MTTTTVSNDQLAKEYVDGVFEELKNQNSHQAEFLQAAEEIFISLVPVFAQHPEYIKANILSRIVEPDRIISFRVAWQDDNNQVQVNRGYRVQYSNVMGPYKGGLRFHPSVNESIIKFLGFEQIFKNALTGQPIGGGKGGSNFNPKGKSDSEIMRFCQAFMTELYRHIGPDVDGPGGDIGVGAREVGYLWGQYKRITKAWESGVLTGKTPGYGGSLARKEATGYGTVYFVEEMLKEVNDSFEDKTVVVSGSGNVSTYAIEKAQAYGAKVVACSDSSGYIYDAEGLDLDVIKEIKEVKGDRISTYVDYRPNATFTEGCTGIWSIPCDIALPCATQNEINGDAARTLISNGVKAIGEGANMPSDLEAINEFLNAGVLFGPAKAANAGGVAVSALEMAQDSSRVFWTFEEVDAKLHQIMKNIYADSKAAADKYGYPGNLVVGANIAGFIKVADGMLAEGIY

SEQ ID NO: 59 - protein, 457 aa, synthetic construct
MTTTTVSNDQLAKEYVDGVFEQLKNQNSHQAEFLQAAEEIFISLVPVFAQHPEYIQANILSRIVEPDRIISFRVAWQDDNNQVQVNRGYRVQYSNVMGPYKGGLRFHPSVNESIIKFLGFEQIFKNALTGQPIGGGKGGSNFNPKGKSDSEIMRFCQAFMTELYRHIGPDVDGPGGDIGVGAREVGYLWGQYKRITKAYESGVLTGKTPGYGGSLARKEATGYGTVYFVEEMLKEVNDSFEDKTVVVSGSGNVSTYAIEKAQAYGAKVVACSDSSGYIYDAEGLDLDVIKEIKEVKGDRISTYVDYRPNATFTEGCTGIWSIPCDIALPCATQNEINGDAARTLISNGVKAIGEGANMPSDLEAINEFLNAGVLFGPAKAANAGGVAVSALEMAQDSSRVFWTFEEVDAKLHQIMKNIYADSKAAADKYGYPGNLVVGANIAGFIKVADGMLAEGIY

SEQ ID NO: 60 - protein, 457 aa, synthetic construct
MTTTTVSNDQLAKEYVDGVFEELKNQNSHQAEFLQAAEEIFISLVPVFAQHPEYIKANILSRIVEPDRIISFRVAWQDDNNQVQVNRGYRVQYSNVMGPYKGGLRFHPSVNESIIKFLGFEQIFKNALTGQPIGGGKGGSNFNPKGKSDSEIMRFCQAFMTELYRHIGPDVDGPGGDIGVGAREVGYLWGQYKRITKAYESGVLTGKTPGYGGSLARKEATGYGTVYFVEEMLKEVNDSFEDKTVVVSGSGNVSTYAIEKAQAYGAKVVACSDSSGYIYDAEGLDLDVIKEIKEVKGDRISTYVDYRPNATFTEGCTGIWSIPCDIALPCATQNEINGDAARTLISNGVKAIGEGANMPSDLEAINEFLNAGVLFGPAKAANAGGVAVSALEMAQDSSRVFWTFEEVDAKLHQIMKNIYADSKAAADKYGYPGNLVVGANIAGFIKVADGMLAEGIY

SEQ ID NO: 61 - protein, 457 aa, synthetic construct
MTTTTVSNDQLAKEYVDGVFEQLKNQNSHQAEFLQAAEEIFISLVPVFAQHPEYIQANILSRIVEPDRIISFRVAWQDDNNQVQVNRGYRVQYSNVMGPYKGGLRFHPSVNESIIKFLGFEQIFKNALTGQPIGGGKGGSNFNPKGKSDSEIMRFCQAFMTELYRHIGPDVDGPGGDIGVGAREVGYLWGQYKRITKAYESGVLTGKTPGYGGSLARKEATGYGTVYFVEEMLKEVNDSFEDKTVVVSGSGNVSTYAIEKAQAYGAKVVACSDSSGYIYDAEGLDLDVIKEIKEVKGDRISTYVDYRPNATFTEGCTGIWSIPCDIALPCATQNEINGDAARTLISNGVKAIGEGANMPSDLEAINEFLNAGVLFGPAKAANAGGVAVSALEMAQDSSRVFWTFEEVDAKLHQIMKNIYRDSKAAADKYGYPGNLVVGANIAGFIKVADGMLAEGIY

SEQ ID NO: 62 - protein, 457 aa, synthetic construct
MTTTTVSNDQLAKEYVDGVFEELKNQNSHQAEFLQAAEEIFISLVPVFAQHPEYIKANILSRIVEPDRIISFRVAWQDDNNQVQVNRGYRVQYSNVMGPYKGGLRFHPSVNESIIKFLGFEQIFKNALTGQPIGGGKGGSNFNPKGKSDSEIMRFCQAFMTELYRHIGPDVDGPGGDIGVGAREVGYLWGQYKRITKAYESGVLTGKTPGYGGSLARKEATGYGTVYFVEEMLKEVNDSFEDKTVVVSGSGNVSTYAIEKAQAYGAKVVACSDSSGYIYDAEGLDLDVIKEIKEVKGDRISTYVDYRPNATFTEGCTGIWSIPCDIALPCATQNEINGDAARTLISNGVKAIGEGANMPSDLEAINEFLNAGVLFGPAKAANAGGVAVSALEMAQDSSRVFWTFEEVDAKLHQIMKNIYRDSKAAADKYGYPGNLVVGANIAGFIKVADGMLAEGIY

SEQ ID NO: 63 - protein, 457 aa, synthetic construct
MTTTTVSNDQLAKEYVDGVFEELKNQNSHQAEFLQAAEEIFISLVPVFAQHPEYIQANILSRIVEPDRIISFRVAWQDDNNQVQVNRGYRVQYSNVMGPYKGGLRFHPSVNESIIKFLGFEQIFKNALTGQPIGGGKGGSNFNPKGKSDSEIMRFCQAFMTELYRHIGPDVDGPGGDIGVGAREVGYLWGQYKRITKAYESGVLTGKTPGYGGSLARKEATGYGTVYFVEEMLKEVNDSFEDKTVVVSGSGNVSTYAIEKAQAYGAKVVACSDSSGYIYDAEGLDLDVIKEIKEVKGDRISTYVDYRPNATFTEGCTGIWSIPCDIALPCATQNEINGDAARTLISNGVKAIGEGANMPSDLEAINEFLNAGVLFGPAKAANAGGVAVSALEMAQDSSRVFWTFEEVDAKLHQIMKNIYADSKAAADKYGYPGNLVVGANIAGFIKVADGMLAEGIY

SEQ ID NO: 64 - protein, 457 aa, synthetic construct
MTTTTVSNDQLAKEYVDGVFEELKNQNSHQAEFLQAAEEIFISLVPVFAQHPEYIQANILSRIVEPDRIISFRVAWQDDNNQVQVNRGYRVQYSNVMGPYKGGLRFHPSVNESIIKFLGFEQIFKNALTGQPIGGGKGGSNFNPKGKSDSEIMRFCQAFMTELYRHIGPDVDGPGGDIGVGAREVGYLWGQYKRITKAWESGVLTGKTPGYGGSLARKEATGYGTVYFVEEMLKEVNDSFEDKTVVVSGSGNVSTYAIEKAQAYGAKVVACSDSSGYIYDAEGLDLDVIKEIKEVKGDRISTYVDYRPNATFTEGCTGIWSIPCDIALPCATQNEINGDAARTLISNGVKAIGEGANMPSDLEAINEFLNAGVLFGPAKAANAGGVAVSALEMAQDSSRVFWTFEEVDAKLHQIMKNIYADSKAAADKYGYPGNLVVGANIAGFIKVADGMLAEGIY

SEQ ID NO: 65 - protein, 457 aa, synthetic construct
MTTTTVSNDQLAKEYVDGVFEELKNQNSHQAEFLQAAEEIFISLVPVFAQHPEYIQANILSRIVEPDRIISFRVAWQDDNNQVQVNRGYRVQYSNVMGPYKGGLRFHPSVNESIIKFLGFEQIFKNALTGQPIGGGKGGSNFNPKGKSDSEIMRFCQAFMTELYRHIGPDVDGPGGDIGVGAREVGYLWGQYKRITKAYESGVLTGKTPGYGGSLARKEATGYGTVYFVEEMLKEVNDSFEDKTVVVSGSGNVSTYAIEKAQAYGAKVVACSDSSGYIYDAEGLDLDVIKEIKEVKGDRISTYVDYRPNATFTEGCTGIWSIPCDIALPCATQNEINGDAARTLISNGVKAIGEGANMPSDLEAINEFLNAGVLFGPAKAANAGGVAVSALEMAQDSSRVFWTFEEVDAKLHQIMKNIYRDSKAAADKYGYPGNLVVGANIAGFIKVADGMLAEGIY

SEQ ID NO: 66 - protein, 457 aa, synthetic construct
MTTTTVSNDQLAKEYVDGVFEELKNQNSHQHEFLQAAEEIFISLVPVFAQHPEYIQANILSRIVEPDRIISFRVAWQDDNNQVQVNRGYRVQYSNVMGPYKGGLRFHPSVNESIIKFLGFEQIFKNALTGQPIGGGKGGSNFNPKGKSDSEIMRFCQAFMTELYRHIGPDVDGPGGDIGVGAREVGYLWGQYKRITKAYESGVLTGKTPGYGGSLARKEATGYGTVYFVEEMLKEVNDSFEDKTVVVSGSGNVSTYAIEKAQAYGAKVVACSDSSGYIYDAEGLDLDVIKEIKEVKGDRISTYVDYRPNATFTEGCTGIWSIPCDIALPCATQNEINGDAARTLISNGVKAIGEGANMPSDLEAINEFLNAGVLFGPAKAANAGGVAVSALEMAQDSSRVFWTFEEVDAKLHQIMKNIYRDSKAAADKYGYPGNLVVGANIAGFIKVADGMLAEGIY

SEQ ID NO: 67 - protein, 457 aa, synthetic construct
MTTTTVSNDQLAKEYVDGVFEELKNQNSHQAEFLQAAEEIFISLVPVFAQHPEYIQANILSRIVEPDRIISFRVAWQDDNNQVQVNRGYRVQYSNVMGPYKGGLRFHPSVNESIIKFLGFEQILKNALTGQPIGGGKGGSNFNPKGKSDSEIMRFCQAFMTELYRHIGPDVDGPGGDIGVGAREVGYLWGQYKRITKAYESGVLTGKTPGYGGSLARKEATGYGTVYFVEEMLKEVNDSFEDKTVVVSGSGNVSTYAIEKAQAYGAKVVACSDSSGYIYDAEGLDLDVIKEIKEVKGDRISTYVDYRPNATFTEGCTGIWSIPCDIALPCATQNEINGDAARTLISNGVKAIGEGANMPSDLEAINEFLNAGVLFGPAKAANAGGVAVSALEMAQDSSRVFWTFEEVDAKLHQIMKNIYRDSKAAADKYGYPGNLVVGANIAGFIKVADGMLAEGIY

SEQ ID NO: 68 - protein, 457 aa, synthetic construct
MTTTTVSNDQLAKEYVDGVFEELKNQNSHQAEFLQAAEEIFISLVPVFAQHPEYIQANILSRIVEPDRIISFRVAWQDDNNQVQVNRGYRVQYSNVMGPYKGGLRFHPSVNESIIKFLGFEQIFKNALTGQPIGGGKGGSNFNPKGKSDSEIMRFCQAFMTELYRHIGPDVDGPGGDIGVGAREVGYLWGQYKRITKAYESGVLTGKTPGYGGSLGRKEATGYGTVYFVEEMLKEVNDSFEDKTVVVSGSGNVSTYAIEKAQAYGAKVVACSDSSGYIYDAEGLDLDVIKEIKEVKGDRISTYVDYRPNATFTEGCTGIWSIPCDIALPCATQNEINGDAARTLISNGVKAIGEGANMPSDLEAINEFLNAGVLFGPAKAANAGGVAVSALEMAQDSSRVFWTFEEVDAKLHQIMKNIYRDSKAAADKYGYPGNLVVGANIAGFIKVADGMLAEGIY

SEQ ID NO: 69 - protein, 457 aa, synthetic construct
MTTTTVSNDQLAKEYVDGVFEELKNQNSHQHEFLQAAEEIFISLVPVFAQHPEYIQANILSRIVEPDRIISFRVAWQDDNNQVQVNRGYRVQYSNVMGPYKGGLRFHPSVNESIIKFLGFEQILKNALTGQPIGGGKGGSNFNPKGKSDSEIMRFCQAFMTELYRHIGPDVDGPGGDIGVGAREVGYLWGQYKRITKAYESGVLTGKTPGYGGSLARKEATGYGTVYFVEEMLKEVNDSFEDKTVVVSGSGNVSTYAIEKAQAYGAKVVACSDSSGYIYDAEGLDLDVIKEIKEVKGDRISTYVDYRPNATFTEGCTGIWSIPCDIALPCATQNEINGDAARTLISNGVKAIGEGANMPSDLEAINEFLNAGVLFGPAKAANAGGVAVSALEMAQDSSRVFWTFEEVDAKLHQIMKNIYRDSKAAADKYGYPGNLVVGANIAGFIKVADGMLAEGIY

SEQ ID NO: 70 - protein, 457 aa, synthetic construct
MTTTTVSNDQLAKEYVDGVFEELKNQNSHQHEFLQAAEEIFISLVPVFAQHPEYIQANILSRIVEPDRIISFRVAWQDDNNQVQVNRGYRVQYSNVMGPYKGGLRFHPSVNESIIKFLGFEQIFKNALTGQPIGGGKGGSNFNPKGKSDSEIMRFCQAFMTELYRHIGPDVDGPGGDIGVGAREVGYLWGQYKRITKAYESGVLTGKTPGYGGSLGRKEATGYGTVYFVEEMLKEVNDSFEDKTVVVSGSGNVSTYAIEKAQAYGAKVVACSDSSGYIYDAEGLDLDVIKEIKEVKGDRISTYVDYRPNATFTEGCTGIWSIPCDIALPCATQNEINGDAARTLISNGVKAIGEGANMPSDLEAINEFLNAGVLFGPAKAANAGGVAVSALEMAQDSSRVFWTFEEVDAKLHQIMKNIYRDSKAAADKYGYPGNLVVGANIAGFIKVADGMLAEGIY

SEQ ID NO: 71 - protein, 457 aa, synthetic construct
MTTTTVSNDQLAKEYVDGVFEELKNQNSHQAEFLQAAEEIFISLVPVFAQHPEYIQANILSRIVEPDRIISFRVAWQDDNNQVQVNRGYRVQYSNVMGPYKGGLRFHPSVNESIIKFLGFEQILKNALTGQPIGGGKGGSNFNPKGKSDSEIMRFCQAFMTELYRHIGPDVDGPGGDIGVGAREVGYLWGQYKRITKAYESGVLTGKTPGYGGSLGRKEATGYGTVYFVEEMLKEVNDSFEDKTVVVSGSGNVSTYAIEKAQAYGAKVVACSDSSGYIYDAEGLDLDVIKEIKEVKGDRISTYVDYRPNATFTEGCTGIWSIPCDIALPCATQNEINGDAARTLISNGVKAIGEGANMPSDLEAINEFLNAGVLFGPAKAANAGGVAVSALEMAQDSSRVFWTFEEVDAKLHQIMKNIYRDSKAAADKYGYPGNLVVGANIAGFIKVADGMLAEGIY

SEQ ID NO: 72 - protein, 457 aa, synthetic construct
MTTTTVSNDQLAKEYVDGVFEELKNQNSHQHEFLQAAEEIFISLVPVFAQHPEYIQANILSRIVEPDRIISFRVAWQDDNNQVQVNRGYRVQYSNVMGPYKGGLRFHPSVNESIIKFLGFEQILKNALTGQPIGGGKGGSNFNPKGKSDSEIMRFCQAFMTELYRHIGPDVDGPGGDIGVGAREVGYLWGQYKRITKAYESGVLTGKTPGYGGSLGRKEATGYGTVYFVEEMLKEVNDSFEDKTVVVSGSGNVSTYAIEKAQAYGAKVVACSDSSGYIYDAEGLDLDVIKEIKEVKGDRISTYVDYRPNATFTEGCTGIWSIPCDIALPCATQNEINGDAARTLISNGVKAIGEGANMPSDLEAINEFLNAGVLFGPAKAANAGGVAVSALEMAQDSSRVFWTFEEVDAKLHQIMKNIYRDSKAAADKYGYPGNLVVGANIAGFIKVADGMLAEGIY

SEQ ID NO: 73 - protein, 457 aa, synthetic construct
MTTTTVSNDQLAKEYVDGVFEELKNQNSHQAEFLQAAEEIFISLVPVFAQHPEYIQANILSRIVEPDRIISFRVAWQDDNNQVQVNRGYRVQYSNVMGPYKGGLRFHPSVNESIIKFLGFEQIFKNALTGQPIGGGKGGSNFNPKGKSDSEIMRFCQAFMTELYRHIGPDVDGPGGDIGVGAREVGYLWGQYKRITKAYESGVLTGKTPGYGGSLARKEATGYGTVYFVEEMLKEVNDSFEDKTVVVSGSGNVSTYAIEKAQAYGAKVVACSDSSGYIYDAEGLDLDVIKEIKEVKGDRISTYVDYRPNATFTEGCTGIWSIPCDIALPCATQNEINGDAARTLISNGVKAIGEGANMPSDLEAINEFLNAGVLFGPAKACNAGGVAVSALEMAQDSSRVFWTFEEVDAKLHQIMKNIYRDSKAAADKYGYPGNLVVGANIAGFIKVADGMLAEGIY

SEQ ID NO: 74 - protein, 457 aa, synthetic construct
MTTTTVSNDQLAKEYVDGVFEELKNQNSHQHEFLQAAEEIFISLVPVFAQHPEYIQANILSRIVEPDRIISFRVAWQDDNNQVQVNRGYRVQYSNVMGPYKGGLRFHPSVNESIIKFLGFEQIFKNALTGQPIGGGKGGSNFNPKGKSDSEIMRFCQAFMTELYRHIGPDVDGPGGDIGVGAREVGYLWGQYKRITKAYESGVLTGKTPGYGGSLARKEATGYGTVYFVEEMLKEVNDSFEDKTVVVSGSGNVSTYAIEKAQAYGAKVVACSDSSGYIYDAEGLDLDVIKEIKEVKGDRISTYVDYRPNATFTEGCTGIWSIPCDIALPCATQNEINGDAARTLISNGVKAIGEGANMPSDLEAINEFLNAGVLFGPAKACNAGGVAVSALEMAQDSSRVFWTFEEVDAKLHQIMKNIYRDSKAAADKYGYPGNLVVGANIAGFIKVADGMLAEGIY

SEQ ID NO: 75 - protein, 457 aa, synthetic construct
MTTTTVSNDQLAKEYVDGVFEELKNQNSHQAEFLQAAEEIFISLVPVFAQHPEYIQANILSRIVEPDRIISFRVAWQDDNNQVQVNRGYRVQYSNVMGPYKGGLRFHPSVNESIIKFLGFEQILKNALTGQPIGGGKGGSNFNPKGKSDSEIMRFCQAFMTELYRHIGPDVDGPGGDIGVGAREVGYLWGQYKRITKAYESGVLTGKTPGYGGSLARKEATGYGTVYFVEEMLKEVNDSFEDKTVVVSGSGNVSTYAIEKAQAYGAKVVACSDSSGYIYDAEGLDLDVIKEIKEVKGDRISTYVDYRPNATFTEGCTGIWSIPCDIALPCATQNEINGDAARTLISNGVKAIGEGANMPSDLEAINEFLNAGVLFGPAKACNAGGVAVSALEMAQDSSRVFWTFEEVDAKLHQIMKNIYRDSKAAADKYGYPGNLVVGANIAGFIKVADGMLAEGIY

SEQ ID NO: 76 - protein, 457 aa, synthetic construct
MTTTTVSNDQLAKEYVDGVFEELKNQNSHQAEFLQAAEEIFISLVPVFAQHPEYIQANILSRIVEPDRIISFRVAWQDDNNQVQVNRGYRVQYSNVMGPYKGGLRFHPSVNESIIKFLGFEQIFKNALTGQPIGGGKGGSNFNPKGKSDSEIMRFCQAFMTELYRHIGPDVDGPGGDIGVGAREVGYLWGQYKRITKAYESGVLTGKTPGYGGSLGRKEATGYGTVYFVEEMLKEVNDSFEDKTVVVSGSGNVSTYAIEKAQAYGAKVVACSDSSGYIYDAEGLDLDVIKEIKEVKGDRISTYVDYRPNATFTEGCTGIWSIPCDIALPCATQNEINGDAARTLISNGVKAIGEGANMPSDLEAINEFLNAGVLFGPAKACNAGGVAVSALEMAQDSSRVFWTFEEVDAKLHQIMKNIYRDSKAAADKYGYPGNLVVGANIAGFIKVADGMLAEGIY

SEQ ID NO: 77 - protein, 457 aa, synthetic construct
MTTTTVSNDQLAKEYVDGVFEELKNQNSHQHEFLQAAEEIFISLVPVFAQHPEYIQANILSRIVEPDRIISFRVAWQDDNNQVQVNRGYRVQYSNVMGPYKGGLRFHPSVNESIIKFLGFEQILKNALTGQPIGGGKGGSNFNPKGKSDSEIMRFCQAFMTELYRHIGPDVDGPGGDIGVGAREVGYLWGQYKRITKAYESGVLTGKTPGYGGSLARKEATGYGTVYFVEEMLKEVNDSFEDKTVVVSGSGNVSTYAIEKAQAYGAKVVACSDSSGYIYDAEGLDLDVIKEIKEVKGDRISTYVDYRPNATFTEGCTGIWSIPCDIALPCATQNEINGDAARTLISNGVKAIGEGANMPSDLEAINEFLNAGVLFGPAKACNAGGVAVSALEMAQDSSRVFWTFEEVDAKLHQIMKNIYRDSKAAADKYGYPGNLVVGANIAGFIKVADGMLAEGIY

SEQ ID NO: 78 - protein, 457 aa, synthetic construct
MTTTTVSNDQLAKEYVDGVFEELKNQNSHQHEFLQAAEEIFISLVPVFAQHPEYIQANILSRIVEPDRIISFRVAWQDDNNQVQVNRGYRVQYSNVMGPYKGGLRFHPSVNESIIKFLGFEQIFKNALTGQPIGGGKGGSNFNPKGKSDSEIMRFCQAFMTELYRHIGPDVDGPGGDIGVGAREVGYLWGQYKRITKAYESGVLTGKTPGYGGSLGRKEATGYGTVYFVEEMLKEVNDSFEDKTVVVSGSGNVSTYAIEKAQAYGAKVVACSDSSGYIYDAEGLDLDVIKEIKEVKGDRISTYVDYRPNATFTEGCTGIWSIPCDIALPCATQNEINGDAARTLISNGVKAIGEGANMPSDLEAINEFLNAGVLFGPAKACNAGGVAVSALEMAQDSSRVFWTFEEVDAKLHQIMKNIYRDSKAAADKYGYPGNLVVGANIAGFIKVADGMLAEGIY

SEQ ID NO: 79 - protein, 457 aa, synthetic construct
MTTTTVSNDQLAKEYVDGVFEELKNQNSHQAEFLQAAEEIFISLVPVFAQHPEYIQANILSRIVEPDRIISFRVAWQDDNNQVQVNRGYRVQYSNVMGPYKGGLRFHPSVNESIIKFLGFEQILKNALTGQPIGGGKGGSNFNPKGKSDSEIMRFCQAFMTELYRHIGPDVDGPGGDIGVGAREVGYLWGQYKRITKAYESGVLTGKTPGYGGSLGRKEATGYGTVYFVEEMLKEVNDSFEDKTVVVSGSGNVSTYAIEKAQAYGAKVVACSDSSGYIYDAEGLDLDVIKEIKEVKGDRISTYVDYRPNATFTEGCTGIWSIPCDIALPCATQNEINGDAARTLISNGVKAIGEGANMPSDLEAINEFLNAGVLFGPAKACNAGGVAVSALEMAQDSSRVFWTFEEVDAKLHQIMKNIYRDSKAAADKYGYPGNLVVGANIAGFIKVADGMLAEGIY

SEQ ID NO: 80 - protein, 457 aa, synthetic construct
MTTTTVSNDQLAKEYVDGVFEELKNQNSHQHEFLQAAEEIFISLVPVFAQHPEYIQANILSRIVEPDRIISFRVAWQDDNNQVQVNRGYRVQYSNVMGPYKGGLRFHPSVNESIIKFLGFEQILKNALTGQPIGGGKGGSNFNPKGKSDSEIMRFCQAFMTELYRHIGPDVDGPGGDIGVGAREVGYLWGQYKRITKAYESGVLTGKTPGYGGSLGRKEATGYGTVYFVEEMLKEVNDSFEDKTVVVSGSGNVSTYAIEKAQAYGAKVVACSDSSGYIYDAEGLDLDVIKEIKEVKGDRISTYVDYRPNATFTEGCTGIWSIPCDIALPCATQNEINGDAARTLISNGVKAIGEGANMPSDLEAINEFLNAGVLFGPAKACNAGGVAVSALEMAQDSSRVFWTFEEVDAKLHQIMKNIYRDSKAAADKYGYPGNLVVGANIAGFIKVADGMLAEGIY